European Patent Application EP 4 631 515 A1, published October 15, 2025. Title: ANTITUMOR TOXINS. Applicant: Fundació Institut D'Investigació Biomèdica De Bellvitge (IDIBELL). The sequence listing filed with the application follows.

SEQUENCE LISTING (33 sequences)

SEQ ID NO: 1 - protein, 338 aa, Bacillus thuringiensis
MYNDKRMCSDPYQGMNKPHYCNCHTYNNSEITGGLQVDLDNQVVETFQSTTDVIREYLMFNELSALSSSPESVRSRFSSIYGTNPDGIALNNETYFNAVKPPITAQYGYYCYKNVGTVQYVNRPTDINPNVILAQDTLTNNTNEPFTTTITITGSFTNTSTVTSSTTTGFKFTSKLSIKKVFEIGGEVSFSTTIGTSETTTETITVSKSVTVTVPAQSRRTIQLTAKIAKESADFSAPITVDGYFGANFPKRVGPGGHYFWFNPARDVLNTTSGTLRGTVTNVSSFDFQTIVQPARSLLDEQQETLEYAIPGDPSGEQLQQMEQRMFFSKCQCPKWGN

SEQ ID NO: 2 - protein, 356 aa, synthetic construct
MGWSCIILFLVATATGVHSYNDKRMCSDPYQGMNKPHYCNCHTYNNSEITGGLQVDLDNQVVETFQSTTDVIREYLMFNELSALSSSPESVRSRFSSIYGTNPDGIALNNETYFNAVKPPITAQYGYYCYKNVGTVQYVNRPTDINPNVILAQDTLTNNTNEPFTTTITITGSFTNTSTVTSSTTTGFKFTSKLSIKKVFEIGGEVSFSTTIGTSETTTETITVSKSVTVTVPAQSRRTIQLTAKIAKESADFSAPITVDGYFGANFPKRVGPGGHYFWFNPARDVLNTTSGTLRGTVTNVSSFDFQTIVQPARSLLDEQQETLEYAIPGDPSGEQLQQMEQRMFFSKCQCPKWGN

SEQ ID NO: 3 - protein, 8 aa, synthetic construct
LEVLFQGM

SEQ ID NO: 4 - protein, 372 aa, synthetic construct
MGWSCIILFLVATATGVHSYNDKRMCSDPYQGMNKPHYCNCHTYNNSEITGGLQVDLDNQVVETFQSTTLEVLFQGMDVIREYLMFNELSALSSSPESVRSRFSSIYGTNPDGIALNNETYFNAVKPPITAQYGYYCYKNVGTVQYVNRPTDINPNVILAQDTLTNNTNEPFTTTITITGSFTNTSTVTSSTTTGFKFTSKLSIKKVFEIGGEVSFSTTIGTSETTTETITVSKSVTVTVPAQSRRTIQLTAKIAKESADFSAPITVDGYFGANFPKRVGPGGHYFWFNPARDVLNTTSGTLRGTVTNVSSFDFQTIVQPARSLLDEQLEVLFQGMQETLEYAIPGDPSGEQLQQMEQRMFFSKCQCPKWGN

SEQ ID NO: 5 - protein, 14 aa, synthetic construct
GGSLSGRSDNHGGS

SEQ ID NO: 6 - protein, 384 aa, synthetic construct
MGWSCIILFLVATATGVHSYNDKRMCSDPYQGMNKPHYCNCHTYNNSEITGGLQVDLDNQVVETFQSTTGGSLSGRSDNHGGSDVIREYLMFNELSALSSSPESVRSRFSSIYGTNPDGIALNNETYFNAVKPPITAQYGYYCYKNVGTVQYVNRPTDINPNVILAQDTLTNNTNEPFTTTITITGSFTNTSTVTSSTTTGFKFTSKLSIKKVFEIGGEVSFSTTIGTSETTTETITVSKSVTVTVPAQSRRTIQLTAKIAKESADFSAPITVDGYFGANFPKRVGPGGHYFWFNPARDVLNTTSGTLRGTVTNVSSFDFQTIVQPARSLLDEQGGSLSGRSDNHGGSQETLEYAIPGDPSGEQLQQMEQRMFFSKCQCPKWGN

SEQ ID NO: 7 - protein, 4 aa, synthetic construct
SGRS

SEQ ID NO: 8 - protein, 5 aa, synthetic construct
SGRSG

SEQ ID NO: 9 - protein, 357 aa, synthetic construct
MGWSCIILFLVATATGVHSYNDKRMCSDPYQGMNKPHYCNCHTYNNSEITGGLQVDLDNQVVETFQSSGRSVIREYLMFNELSALSSSPESVRSRFSSIYGTNPDGIALNNETYFNAVKPPITAQYGYYCYKNVGTVQYVNRPTDINPNVILAQDTLTNNTNEPFTTTITITGSFTNTSTVTSSTTTGFKFTSKLSIKKVFEIGGEVSFSTTIGTSETTTETITVSKSVTVTVPAQSRRTIQLTAKIAKESADFSAPITVDGYFGANFPKRVGPGGHYFWFNPARDVLNTTSGTLRGTVTNVSSFDFQTIVQPARSLLSGRSGTLEYAIPGDPSGEQLQQMEQRMFFSKCQCPKWGN

SEQ ID NO: 10 - protein, 5 aa, synthetic construct
QRLRR

SEQ ID NO: 11 - protein, 360 aa, synthetic construct
MGWSCIILFLVATATGVHSYNDKRMCSDPYQGMNKPHYCNCHTYNNSEITGGLQVDLDNQVVETFQSTQRLRRDVIREYLMFNELSALSSSPESVRSRFSSIYGTNPDGIALNNETYFNAVKPPITAQYGYYCYKNVGTVQYVNRPTDINPNVILAQDTLTNNTNEPFTTTITITGSFTNTSTVTSSTTTGFKFTSKLSIKKVFEIGGEVSFSTTIGTSETTTETITVSKSVTVTVPAQSRRTIQLTAKIAKESADFSAPITVDGYFGANFPKRVGPGGHYFWFNPARDVLNTTSGTLRGTVTNVSSFDFQTIVQPARSLLDEQQETLEYAIPGDPSGEQLQQMEQRMFFSKCQCPKWGN

SEQ ID NO: 12 - protein, 4 aa, synthetic construct
RRKR

SEQ ID NO: 13 - protein, 364 aa, synthetic construct
MGWSCIILFLVATATGVHSYNDKRMCSDPYQGMNKPHYCNCHTYNNSEITGGLQVDLDNQVVETFQSTQRLRRDVIREYLMFNELSALSSSPESVRSRFSSIYGTNPDGIALNNETYFNAVKPPITAQYGYYCYKNVGTVQYVNRPTDINPNVILAQDTLTNNTNEPFTTTITITGSFTNTSTVTSSTTTGFKFTSKLSIKKVFEIGGEVSFSTTIGTSETTTETITVSKSVTVTVPAQSRRTIQLTAKIAKESADFSAPITVDGYFGANFPKRVGPGGHYFWFNPARDVLNTTSGTLRGTVTNVSSFDFQTIVQPARSLLDEQQRRKRETLEYAIPGDPSGEQLQQMEQRMFFSKCQCPKWGN

SEQ ID NO: 14 - protein, 304 aa, Bacillus thuringiensis
MYYTTQVTGGFQADLNNQVVETFQPSTNVIQEYLTFNDLPALGSSPQSVRSRFSSIYGTNPDGIALNNETYFSAVQPPITVQYGHYCYKNVGTVQYVNRPTDINPNVILAQDTLTNNTNEPFTTTITLTGSWTKSSTVTSSTTTGLKITTKLSIKKVFEIGGEVSFSTTIGSSEATSETFTVSKAVTVTVPAQSRRNIQLTAKIARESADFSAPITVDGYFGANFPRRVGPGGHYFWFNPARDVLNATSGTLRGTVTNVSSFDFQTVVQPAYSLLAEQQEALESAISGDPSEEQLKQIQQTIGL

SEQ ID NO: 15 - protein, 330 aa, synthetic construct
MGWSCIILFLVATATGVHSYYTTQVTGGFQADLNNQVVETFQPSTRLRRNVIQEYLTFNDLPALGSSPQSVRSRFSSIYGTNPDGIALNNETYFSAVQPPITVQYGHYCYKNVGTVQYVNRPTDINPNVILAQDTLTNNTNEPFTTTITLTGSWTKSSTVTSSTTTGLKITTKLSIKKVFEIGGEVSFSTTIGSSEATSETFTVSKAVTVTVPAQSRRNIQLTAKIARESADFSAPITVDGYFGANFPRRVGPGGHYFWFNPARDVLNATSGTLRGTVTNVSSFDFQTVVQPAYSLLAEQQRRKREALESAISGDPSEEQLKQIQQTIGL

SEQ ID NO: 16 - protein, 4 aa, synthetic construct
RLRR

SEQ ID NO: 17 - protein, 19 aa, synthetic construct
MGWSCIILFLVATATGVHS

SEQ ID NO: 18 - protein, 51 aa, synthetic construct
MYNDKRMCSDPYQGMNKPHYCNCHTYNNSEITGGLQVDLDNQVVETFQSTT

SEQ ID NO: 19 - protein, 36 aa, synthetic construct
QETLEYAIPGDPSGEQLQQMEQRMFFSKCQCPKWGN

SEQ ID NO: 20 - protein, 338 aa, Bacillus thuringiensis
MYNDKRMCSDPYQGMNKPHYCNCHTYNNSEITGGLQVDLDNQVAETFQSTTDVIREYLMFNELSALSSSPESVRSRFFSIYGTNPDGIALNNETYFNAVKPPITAQYGYYCYKNVGTVQYVNRPTDINPNVILAQDTLTNNTNEPFTTTITITGSFTNTSTVTSSTTTGFKFTSKLSIKKVFEIGGEVSFSTTIGTSETTTETITVSKSVTVTVPAQSRRTIQLTAKIAKESADFSAPITVDGYFGANFPKRVGPGGHYYWFNPARDVLNTTSGTLRGTVTNVSSFDFQTIVQPARSLLDEQQETLEYAIPGDPSGEQLQQMEQRMFFSQCQCPKWGN

SEQ ID NO: 21 - protein, 6 aa, synthetic construct
HSSKLQ

SEQ ID NO: 22 - protein, 5 aa, synthetic construct
PLGLA

SEQ ID NO: 23 - protein, 4 aa, synthetic construct
IGGL

SEQ ID NO: 24 - protein, 6 aa, synthetic construct
PLGLGL

SEQ ID NO: 25 - protein, 6 aa, synthetic construct
PLGMTS

SEQ ID NO: 26 - protein, 6 aa, synthetic construct
PLGLWA

SEQ ID NO: 27 - protein, 8 aa, synthetic construct
LSGRSDNH

SEQ ID NO: 28 - protein, 5 aa, synthetic construct
DDDDK

SEQ ID NO: 29 - protein, 5 aa, synthetic construct
IEDGR

SEQ ID NO: 30 - protein, 6 aa, synthetic construct
LVPRGS

SEQ ID NO: 31 - protein, 7 aa, synthetic construct
ENLYFQG

SEQ ID NO: 32 - protein, 8 aa, synthetic construct
LEVLFQGP

SEQ ID NO: 33 - protein, 5 aa, synthetic construct
DVIRE